European Patent Specification EP 3 784 774 B1, published November 19, 2025. Title: METHODS OF PRODUCING T CELL POPULATIONS USING HYDROXYCITRIC ACID AND/OR A SALT THEREOF. Applicant: THE UNITED STATES OF AMERICA, AS REPRESENTED BY THE SECRETARY, DEPARTMENT OF HEALTH  AND HUMAN SERVICES. The sequence listing filed with the application follows.

SEQUENCE LISTING (2 sequences)

SEQ ID NO: 1 - DNA, 22 bp, Artificial Sequence
  synthetic
ggagccttcgatcaggtataaa

SEQ ID NO: 2 - DNA, 21 bp, Artificial Sequence
  synthetic
ctcaagtcagagggtccaaag